European Patent Application EP 4 678 194 A1, published January 14, 2026. Title: Therapeutic application of 64Cu-labelled peptide conjugate for site-specific uPAR-targeting. Applicant: Curasight. Application EP. The sequence listing filed with the application follows.

SEQUENCE LISTING (18 sequences)

SEQ ID NO: 1 - protein, 9 aa, synthetic construct
  SITE 2: note = [beta]-cyclohexyl-L-alanine
  SITE 1: note = D-aspartic acid
  SITE 4: note = D-serine
  SITE 5: note = D-arginine
DXFSRYLWS

SEQ ID NO: 2 - protein, 10 aa, synthetic construct
  SITE 3: note = [beta]-cyclohexyl-L-alanine
  SITE 5: note = D-serine
SLXFSQYLWS

SEQ ID NO: 3 - protein, 9 aa, synthetic construct
  SITE 1: note = D-glutamic acid
  SITE 2: note = [beta]-cyclohexyl-L-alanine
  SITE 4: note = D-serine
  SITE 5: note = D-tyrosine
EXFSYYLWS

SEQ ID NO: 4 - protein, 9 aa, synthetic construct
  SITE 2: note = [beta]-cyclohexyl-L-alanine
  SITE 4: note = D-serine
  SITE 5: note = D-arginine
DXFSRYLWS

SEQ ID NO: 5 - protein, 9 aa, synthetic construct
  SITE 2: note = [beta]-cyclohexyl-L-alanine
  SITE 5: note = D-arginine
DXFSRYLWS

SEQ ID NO: 6 - protein, 9 aa, synthetic construct
  SITE 1: note = D-aspartic acid
  SITE 2: note = [beta]-cyclohexyl-L-alanine
  SITE 5: note = D-arginine
DXFSRYLWS

SEQ ID NO: 7 - protein, 9 aa, synthetic construct
  SITE 1: note = D-threonine
  SITE 2: note = [beta]-cyclohexyl-L-alanine
  SITE 4: note = D-serine
  SITE 5: note = D-arginine
TXFSRYLWS

SEQ ID NO: 8 - protein, 9 aa, synthetic construct
  SITE 1: note = D-aspartic acid
  SITE 2: note = [beta]-cyclohexyl-L-alanine
  SITE 4: note = D-serine
  SITE 5: note = D-arginine
  SITE 8: note = [beta]-2-naphthyl-L-alanine
DXFSRYLXS

SEQ ID NO: 9 - protein, 9 aa, synthetic construct
  SITE 2: note = [beta]-cyclohexyl-L-alanine
  SITE 4: note = D-serine
DXFSRYLWS

SEQ ID NO: 10 - protein, 9 aa, synthetic construct
  SITE 2: note = [beta]-cyclohexyl-L-alanine
  SITE 4: note = D-serine
  SITE 5: note = D-arginine
  SITE 8: note = [beta]-1-naphthyl-L-alanine
DXFSRYLXS

SEQ ID NO: 11 - protein, 9 aa, synthetic construct
  SITE 1: note = D-glutamic acid
  SITE 2: note = [beta]-cyclohexyl-L-alanine
  SITE 4: note = D-serine
EXFSYYLWS

SEQ ID NO: 12 - protein, 9 aa, synthetic construct
  SITE 2: note = [beta]-cyclohexyl-L-alanine
  SITE 4: note = D-serine
  SITE 5: note = D-arginine
  SITE 9: note = D-histidine
DXFSRLLWH

SEQ ID NO: 13 - protein, 9 aa, synthetic construct
  SITE 2: note = [beta]-cyclohexyl-L-alanine
  SITE 4: note = D-serine
  SITE 5: note = D-arginine
  SITE 6: note = [beta]-cyclohexyl-L-alanine
DXFSRXLWI

SEQ ID NO: 14 - protein, 9 aa, synthetic construct
  SITE 2: note = [beta]-cyclohexyl-L-alanine
  SITE 4: note = D-serine
  SITE 5: note = D-arginine
  SITE 8: note = [beta]-1-naphthyl-L-alanine
  SITE 9: note = D-histidine
DXFSRYLXH

SEQ ID NO: 15 - protein, 9 aa, synthetic construct
  SITE 2: note = [beta]-cyclohexyl-L-alanine
  SITE 4: note = D-serine
  SITE 5: note = D-arginine
  SITE 6: note = N-(2,3-dimethoxybenzyl)glycine
  SITE 7: note = D-phenylalanine
  SITE 8: note = N-(3-indolylethyl)glycine
  SITE 9: note = N-(2-methoxyethyl)glycine
DXFSRXFXX

SEQ ID NO: 16 - protein, 9 aa, synthetic construct
  SITE 2: note = [beta]-cyclohexyl-L-alanine
  SITE 4: note = D-serine
  SITE 5: note = D-arginine
  SITE 6: note = N-(2,3-dimethoxybenzyl)glycine
  SITE 7: note = D-phenylalanine
  SITE 8: note = N-benzylglycine
  SITE 9: note = N-(2[beta]thoxyethyl)glycine
DXFSRXFXX

SEQ ID NO: 17 - protein, 9 aa, synthetic construct
  SITE 2: note = [beta]-cyclohexyl-L-alanine
  SITE 4: note = D-serine
  SITE 5: note = D-arginine
  SITE 6: note = N-(2,3-dimethoxybenzyl)glycine
  SITE 7: note = D-phenylalanine
  SITE 8: note = N-(methylnaphthalyl)glycine
  SITE 9: note = N-(2-methoxyethyl)glycine
DXFSRXFXX

SEQ ID NO: 18 - protein, 9 aa, synthetic construct
  SITE 2: note = [beta]-cyclohexyl-L-alanine
  SITE 4: note = D-serine
  SITE 5: note = D-arginine
  SITE 6: note = N-(2,3-dimethoxybenzyl)glycine
  SITE 7: note = D-phenylalanine
  SITE 8: note = N-(2,3-dimethoxybenzyl)glycine
DXFSRXFXI